European Patent Application EP 4 685 162 A1, published January 28, 2026. Title: HUMAN ANTI-FV ANTIBODY, THERAPEUTIC AND DIAGNOSTIC APPLICATIONS THEREOF. Applicant: CEINGE BIOTECNOLOGIE AVANZATE_FRANCO SALVATORE S.C. A R.L. Application EP. The sequence listing filed with the application follows.

SEQUENCE LISTING (16 sequences)

SEQ ID NO: 1 - protein, 12 aa, Homo sapiens
GFTFSSYAMSWV

SEQ ID NO: 2 - protein, 12 aa, Homo sapiens
GSGGSTYYADSV

SEQ ID NO: 3 - protein, 6 aa, Homo sapiens
GRIRRF

SEQ ID NO: 4 - protein, 9 aa, Homo sapiens
QGDSLRSYY

SEQ ID NO: 5 - protein, 4 aa, Homo sapiens
KNNR

SEQ ID NO: 6 - protein, 11 aa, Homo sapiens
NSRDSSGNHVV

SEQ ID NO: 7 - protein, 115 aa, Homo sapiens
EVQLVESGGGLVQPGGSLRLSCAASGFTFSSYAMSWVRQAPGKGLEWVSAISGSGGSTYYADSVKGRFTISRDNSKNTLYLQMNSLRAEDTAVYYCARGRIRRFWGQGTLVTVSR

SEQ ID NO: 8 - protein, 110 aa, Homo sapiens
ELTQDPAVSVALGQTVRITCQGDSLRSYYASWYQQKPGQAPVLVIYGKNNRPSGIPDRFSGSSSGNTASLTITGAQAEDEADYYCNSRDSSGNHVVFGGGTKLTVLGAAA

SEQ ID NO: 9 - DNA, 35 bp, Homo sapiens
  source 1..35: mol_type = other DNA
ggattcacctttagcagctatgccatgagctgggt

SEQ ID NO: 10 - DNA, 36 bp, Homo sapiens
  source 1..36: mol_type = other DNA
ggtagtggtggtagcacatactacgcagactccgtg

SEQ ID NO: 11 - DNA, 19 bp, Homo sapiens
  source 1..19: mol_type = other DNA
aggtaggattaggcggttt

SEQ ID NO: 12 - DNA, 30 bp, Homo sapiens
  source 1..30: mol_type = other DNA
ccaaggagacagcctcagaagctattatgc

SEQ ID NO: 13 - DNA, 15 bp, Homo sapiens
  source 1..15: mol_type = other DNA
taaaaacaaccggcc

SEQ ID NO: 14 - DNA, 36 bp, Homo sapiens
  source 1..36: mol_type = other DNA
taactcccgggacagcagtggtaaccatgtggtatt

SEQ ID NO: 15 - DNA, 347 bp, Homo sapiens
  source 1..347: mol_type = other DNA
ccgaggtgcagctggtggagtctgggggaggcttggtacagcctggggggtccctgagactctcctgtgcagcctctggattcacctttagcagctatgccatgagctgggtccgccaggctccagggaaggggctggagtgggtctcagctattagtggtagtggtggtagcacatactacgcagactccgtgaagggccggttcaccatctccagagacaattccaagaacacgctgtatctgcaaatgaacagcctgagagccgaggacacggccgtgtattactgtgcaagaggtaggattaggcggttttggggccaaggtaccctggtcaccgtgtcgaga

SEQ ID NO: 16 - DNA, 334 bp, Homo sapiens
  source 1..334: mol_type = other DNA
gtctgagctgactcaggaccctgctgtgtctgtggccttgggacagacagtcaggatcacatgccaaggagacagcctcagaagctattatgcaagctggtaccagcagaagccaggacaggcccctgtacttgtcatctatggtaaaaacaaccggccctcagggatcccagaccgattctctggctccagctcaggaaacacagcttccttgaccatcactggggctcaggcggaagatgaggctgactattactgtaactcccgggacagcagtggtaaccatgtggtattcggcggagggaccaagctgaccgtcctaggtgcggccgca